European Patent Application EP 4 582 445 A1, published July 9, 2025. Title: 抗人补体C5抗体以及其融合蛋白. Applicant: 天辰生物医药（苏州）有限公司. The sequence listing filed with the application follows.

SEQUENCE LISTING (70 sequences)

SEQ ID NO: 1 - protein, 381 aa, artificial sequence
MTVARPSVPAALPLLGELPRLLLLVLLCLPAVWGDCGLPPDVPNAQPALEGRTSFPEDTVITYKCEESFVKIPGEKDSVICLKGSQWSDIEEFCNRSCEVPTRLNSASLKQPYITQNYFPVGTVVEYECRPGYRREPSLSPKLTCLQNLKWSTAVEFCKKKSCPNPGEIRNGQIDVPGGILFGATISFSCNTGYKLFGSTSSFCLISGSSVQWSDPLPECREIYCPAPPQIDNGIIQGERDHYGYRQSVTYACNKGFTMIGEHSIYCTVNNDEGEWSGPPPECRGKSLTSKVPPTVQKPTTVNVPTTEVSPTSQKTTTKTTTPNAQATRSTPVSRTTKHFHETTPNKGSGTTSGTTRLLSGHTCFTLTGLLGTLVTMGLLT

SEQ ID NO: 2 - DNA, 1146 bp, artificial sequence
  source 1..1146: mol_type = other DNA
atgaccgtcgcgcggccgagcgtgcccgcggcgctgcccctcctcggggagctgccccggctgctgctgctggtgctgttgtgcctgccggccgtgtggggtgactgtggccttcccccagatgtacctaatgcccagccagctttggaaggccgtacaagttttcccgaggatactgtaataacgtacaaatgtgaagaaagctttgtgaaaattcctggcgagaaggactcagtgatctgccttaagggcagtcaatggtcagatattgaagagttctgcaatcgtagctgcgaggtgccaacaaggctaaattctgcatccctcaaacagccttatatcactcagaattattttccagtcggtactgttgtggaatatgagtgccgtccaggttacagaagagaaccttctctatcaccaaaactaacttgccttcagaatttaaaatggtccacagcagtcgaattttgtaaaaagaaatcatgccctaatccgggagaaatacgaaatggtcagattgatgtaccaggtggcatattatttggtgcaaccatctccttctcatgtaacacagggtacaaattatttggctcgacttctagtttttgtcttatttcaggcagctctgtccagtggagtgacccgttgccagagtgcagagaaatttattgtccagcaccaccacaaattgacaatggaataattcaaggggaacgtgaccattatggatatagacagtctgtaacgtatgcatgtaataaaggattcaccatgattggagagcactctatttattgtactgtgaataatgatgaaggagagtggagtggcccaccacctgaatgcagaggaaaatctctaacttccaaggtcccaccaacagttcagaaacctaccacagtaaatgttccaactacagaagtctcaccaacttctcagaaaaccaccacaaaaaccaccacaccaaatgctcaagcaacacggagtacacctgtttccaggacaaccaagcattttcatgaaacaaccccaaataaaggaagtggaaccacttcaggtactacccgtcttctatctgggcacacgtgtttcacgttgacaggtttgcttgggacgctagtaaccatgggcttgctgacttag

SEQ ID NO: 3 - protein, 1231 aa, artificial sequence
MRLLAKIICLMLWAICVAEDCNELPPRRNTEILTGSWSDQTYPEGTQAIYKCRPGYRSLGNVIMVCRKGEWVALNPLRKCQKRPCGHPGDTPFGTFTLTGGNVFEYGVKAVYTCNEGYQLLGEINYRECDTDGWTNDIPICEVVKCLPVTAPENGKIVSSAMEPDREYHFGQAVRFVCNSGYKIEGDEEMHCSDDGFWSKEKPKCVEISCKSPDVINGSPISQKIIYKENERFQYKCNMGYEYSERGDAVCTESGWRPLPSCEEKSCDNPYIPNGDYSPLRIKHRTGDEITYQCRNGFYPATRGNTAKCTSTGWIPAPRCTLKPCDYPDIKHGGLYHENMRRPYFPVAVGKYYSYYCDEHFETPSGSYWDHIHCTQDGWSPAVPCLRKCYFPYLENGYNQNYGRKFVQGKSIDVACHPGYALPKAQTTVTCMENGWSPTPRCIRVKTCSKSSIDIENGFISESQYTYALKEKAKYQCKLGYVTADGETSGSITCGKDGWSAQPTCIKSCDIPVFMNARTKNDFTWFKLNDTLDYECHDGYESNTGSTTGSIVCGYNGWSDLPICYERECELPKIDVHLVPDRKKDQYKVGEVLKFSCKPGFTIVGPNSVQCYHFGLSPDLPICKEQVQSCGPPPELLNGNVKEKTKEEYGHSEVVEYYCNPRFLMKGPNKIQCVDGEWTTLPVCIVEESTCGDIPELEHGWAQLSSPPYYYGDSVEFNCSESFTMIGHRSITCIHGVWTQLPQCVAIDKLKKCKSSNLIILEEHLKNKKEFDHNSNIRYRCRGKEGWIHTVCINGRWDPEVNCSMAQIQLCPPPPQIPNSHNMTTTLNYRDGEKVSVLCQENYLIQEGEEITCKDGRWQSIPLCVEKIPCSQPPQIEHGTINSSRSSQESYAHGTKLSYTCEGGFRISEENETTCYMGKWSSPPQCEGLPCKSPPEISHGVVAHMSDSYQYGEEVTYKCFEGFGIDGPAIAKCLGEKWSHPPSCIKTDCLSLPSFENAIPMGEKKDVYKAGEQVTYTCATYYKMDGASNVTCINSRWTGRPTCRDTSCVNPPTVQNAYIVSRQMSKYPSGERVRYQCRSPYEMFGDEEVMCLNGNWTEPPQCKDSTGKCGPPPPIDNGDITSFPLSVYAPASSVEYQCQNLYQLEGNKRITCRNGQWSEPPKCLHPCVISREIMENYNIALRWTAKQKLYSRTGESVEFVCKRGYRLSSRSHTLRTTCWDGKLEYPTCAKR

SEQ ID NO: 4 - DNA, 3696 bp, artificial sequence
  source 1..3696: mol_type = other DNA
atgagacttctagcaaagattatttgccttatgttatgggctatttgtgtagcagaagattgcaatgaacttcctccaagaagaaatacagaaattctgacaggttcctggtctgaccaaacatatccagaaggcacccaggctatctataaatgccgccctggatatagatctcttggaaatgtaataatggtatgcaggaagggagaatgggttgctcttaatccattaaggaaatgtcagaaaaggccctgtggacatcctggagatactccttttggtacttttacccttacaggaggaaatgtgtttgaatatggtgtaaaagctgtgtatacatgtaatgaggggtatcaattgctaggtgagattaattaccgtgaatgtgacacagatggatggaccaatgatattcctatatgtgaagttgtgaagtgtttaccagtgacagcaccagagaatggaaaaattgtcagtagtgcaatggaaccagatcgggaataccattttggacaagcagtacggtttgtatgtaactcaggctacaagattgaaggagatgaagaaatgcattgttcagacgatggtttttggagtaaagagaaaccaaagtgtgtggaaatttcatgcaaatccccagatgttataaatggatctcctatatctcagaagattatttataaggagaatgaacgatttcaatataaatgtaacatgggttatgaatacagtgaaagaggagatgctgtatgcactgaatctggatggcgtccgttgccttcatgtgaagaaaaatcatgtgataatccttatattccaaatggtgactactcacctttaaggattaaacacagaactggagatgaaatcacgtaccagtgtagaaatggtttttatcctgcaacccggggaaatacagcaaaatgcacaagtactggctggatacctgctccgagatgtaccttgaaaccttgtgattatccagacattaaacatggaggtctatatcatgagaatatgcgtagaccatactttccagtagctgtaggaaaatattactcctattactgtgatgaacattttgagactccgtcaggaagttactgggatcacattcattgcacacaagatggatggtcgccagcagtaccatgcctcagaaaatgttattttccttatttggaaaatggatataatcaaaatcatggaagaaagtttgtacagggtaaatctatagacgttgcctgccatcctggctacgctcttccaaaagcgcagaccacagttacatgtatggagaatggctggtctcctactcccagatgcatccgtgtcaaaacatgttccaaatcaagtatagatattgagaatgggtttatttctgaatctcagtatacatatgccttaaaagaaaaagcgaaatatcaatgcaaactaggatatgtaacagcagatggtgaaacatcaggatcaattacatgtgggaaagatggatggtcagctcaacccacgtgcattaaatcttgtgatatcccagtatttatgaatgccagaactaaaaatgacttcacatggtttaagctgaatgacacattggactatgaatgccatgatggttatgaaagcaatactggaagcaccactggttccatagtgtgtggttacaatggttggtctgatttacccatatgttatgaaagagaatgcgaacttcctaaaatagatgtacacttagttcctgatcgcaagaaagaccagtataaagttggagaggtgttgaaattctcctgcaaaccaggatttacaatagttggacctaattccgttcagtgctaccactttggattgtctcctgacctcccaatatgtaaagagcaagtacaatcatgtggtccacctcctgaactcctcaatgggaatgttaaggaaaaaacgaaagaagaatatggacacagtgaagtggtggaatattattgcaatcctagatttctaatgaagggacctaataaaattcaatgtgttgatggagagtggacaactttaccagtgtgtattgtggaggagagtacctgtggagatatacctgaacttgaacatggctgggcccagctttcttcccctccttattactatggagattcagtggaattcaattgctcagaatcatttacaatgattggacacagatcaattacgtgtattcatggagtatggacccaacttccccagtgtgtggcaatagataaacttaagaagtgcaaatcatcaaatttaattatacttgaggaacatttaaaaaacaagaaggaattcgatcataattctaacataaggtacagatgtagaggaaaagaaggatggatacacacagtctgcataaatggaagatgggatccagaagtgaactgctcaatggcacaaatacaattatgcccacctccacctcagattcccaattctcacaatatgacaaccacactgaattatcgggatggagaaaaagtatctgttctttgccaagaaaattatctaattcaggaaggagaagaaattacatgcaaagatggaagatggcagtcaataccactctgtgttgaaaaaattccatgttcacaaccacctcagatagaacacggaaccattaattcatccaggtcttcacaagaaagttatgcacatgggactaaattgagttatacttgtgagggtggtttcaggatatctgaagaaaatgaaacaacatgctacatgggaaaatggagttctccacctcagtgtgaaggccttccttgtaaatctccacctgagatttctcatggtgttgtagctcacatgtcagacagttatcagtatggagaagaagttacgtacaaatgttttgaaggttttggaattgatgggcctgcaattgcaaaatgcttaggagaaaaatggtctcaccctccatcatgcataaaaacagattgtctcagtttacctagctttgaaaatgccatacccatgggagagaagaaggatgtgtataaggcgggtgagcaagtgacttacacttgtgcaacatattacaaaatggatggagccagtaatgtaacatgcattaatagcagatggacaggaaggccaacatgcagagacacctcctgtgtgaatccgcccacagtacaaaatgcttatatagtgtcgagacagatgagtaaatatccatctggtgagagagtacgttatcaatgtaggagcccttatgaaatgtttggggatgaagaagtgatgtgtttaaatggaaactggacggaaccacctcaatgcaaagattctacaggaaaatgtgggccccctccacctattgacaatggggacattacttcattcccgttgtcagtatatgctccagcttcatcagttgagtaccaatgccagaacttgtatcaacttgagggtaacaagcgaataacatgtagaaatggacaatggtcagaaccaccaaaatgcttacatccgtgtgtaatatcccgagaaattatggaaaattataacatagcattaaggtggacagccaaacagaagctttattcgagaacaggtgaatcagttgaatttgtgtgtaaacggggatatcgtctttcatcacgttctcacacattgcgaacaacatgttgggatgggaaactggagtatccaacttgtgcaaaaagatag

SEQ ID NO: 5 - protein, 449 aa, artificial sequence
MRLLAKIICLMLWAICVAEDCNELPPRRNTEILTGSWSDQTYPEGTQAIYKCRPGYRSLGNVIMVCRKGEWVALNPLRKCQKRPCGHPGDTPFGTFTLTGGNVFEYGVKAVYTCNEGYQLLGEINYRECDTDGWTNDIPICEVVKCLPVTAPENGKIVSSAMEPDREYHFGQAVRFVCNSGYKIEGDEEMHCSDDGFWSKEKPKCVEISCKSPDVINGSPISQKIIYKENERFQYKCNMGYEYSERGDAVCTESGWRPLPSCEEKSCDNPYIPNGDYSPLRIKHRTGDEITYQCRNGFYPATRGNTAKCTSTGWIPAPRCTLKPCDYPDIKHGGLYHENMRRPYFPVAVGKYYSYYCDEHFETPSGSYWDHIHCTQDGWSPAVPCLRKCYFPYLENGYNQNYGRKFVQGKSIDVACHPGYALPKAQTTVTCMENGWSPTPRCIRVSFTL

SEQ ID NO: 6 - DNA, 1350 bp, artificial sequence
  source 1..1350: mol_type = other DNA
atgagacttctagcaaagattatttgccttatgttatgggctatttgtgtagcagaagattgcaatgaacttcctccaagaagaaatacagaaattctgacaggttcctggtctgaccaaacatatccagaaggcacccaggctatctataaatgccgccctggatatagatctcttggaaatgtaataatggtatgcaggaagggagaatgggttgctcttaatccattaaggaaatgtcagaaaaggccctgtggacatcctggagatactccttttggtacttttacccttacaggaggaaatgtgtttgaatatggtgtaaaagctgtgtatacatgtaatgaggggtatcaattgctaggtgagattaattaccgtgaatgtgacacagatggatggaccaatgatattcctatatgtgaagttgtgaagtgtttaccagtgacagcaccagagaatggaaaaattgtcagtagtgcaatggaaccagatcgggaataccattttggacaagcagtacggtttgtatgtaactcaggctacaagattgaaggagatgaagaaatgcattgttcagacgatggtttttggagtaaagagaaaccaaagtgtgtggaaatttcatgcaaatccccagatgttataaatggatctcctatatctcagaagattatttataaggagaatgaacgatttcaatataaatgtaacatgggttatgaatacagtgaaagaggagatgctgtatgcactgaatctggatggcgtccgttgccttcatgtgaagaaaaatcatgtgataatccttatattccaaatggtgactactcacctttaaggattaaacacagaactggagatgaaatcacgtaccagtgtagaaatggtttttatcctgcaacccggggaaatacagcaaaatgcacaagtactggctggatacctgctccgagatgtaccttgaaaccttgtgattatccagacattaaacatggaggtctatatcatgagaatatgcgtagaccatactttccagtagctgtaggaaaatattactcctattactgtgatgaacattttgagactccgtcaggaagttactgggatcacattcattgcacacaagatggatggtcgccagcagtaccatgcctcagaaaatgttattttccttatttggaaaatggatataatcaaaatcatggaagaaagtttgtacagggtaaatctatagacgttgcctgccatcctggctacgctcttccaaaagcgcagaccacagttacatgtatggagaatggctggtctcctactcccagatgcatccgtgtcagctttaccctctga

SEQ ID NO: 7 - protein, 62 aa, artificial sequence
KSCPNPGEIRNGQIDVPGGILFGATISFSCNTGYKLFGSTSSFCLISGSSVQWSDPLPECRE

SEQ ID NO: 8 - protein, 60 aa, artificial sequence
CPNPGEIRNGQIDVPGGILFGATISFSCNTGYKLFGSTSSFCLISGSSVQWSDPLPECRE

SEQ ID NO: 9 - protein, 63 aa, artificial sequence
IYCPAPPQIDNGIIQGERDHYGYRQSVTYACNKGFTMIGEHSIYCTVNNDEGEWSGPPPECRG

SEQ ID NO: 10 - protein, 125 aa, artificial sequence
KSCPNPGEIRNGQIDVPGGILFGATISFSCNTGYKLFGSTSSFCLISGSSVQWSDPLPECREIYCPAPPQIDNGIIQGERDHYGYRQSVTYACNKGFTMIGEHSIYCTVNNDEGEWSGPPPECRG

SEQ ID NO: 11 - protein, 123 aa, artificial sequence
CPNPGEIRNGQIDVPGGILFGATISFSCNTGYKLFGSTSSFCLISGSSVQWSDPLPECREIYCPAPPQIDNGIIQGERDHYGYRQSVTYACNKGFTMIGEHSIYCTVNNDEGEWSGPPPECRG

SEQ ID NO: 12 - protein, 66 aa, artificial sequence
EDCNELPPRRNTEILTGSWSDQTYPEGTQAIYKCRPGYRSLGNVIMVCRKGEWVALNPLRKCQKRP

SEQ ID NO: 13 - protein, 64 aa, artificial sequence
EDCNELPPRRNTEILTGSWSDQTYPEGTQAIYKCRPGYRSLGNVIMVCRKGEWVALNPLRKCQK

SEQ ID NO: 14 - protein, 66 aa, artificial sequence
EDCNELPPRRNTEILTGSWSDQTYPEGTQAIYKCRPGYRSLGNIIMVCRKGEWVALNPLRKCQKRP

SEQ ID NO: 15 - protein, 64 aa, artificial sequence
EDCNELPPRRNTEILTGSWSDQTYPEGTQAIYKCRPGYRSLGNIIMVCRKGEWVALNPLRKCQK

SEQ ID NO: 16 - protein, 7 aa, artificial sequence
GHHHHHH

SEQ ID NO: 17 - protein, 19 aa, artificial sequence
MGWSCIILFLVATATGVHS

SEQ ID NO: 18 - protein, 189 aa, artificial sequence
EDCNELPPRRNTEILTGSWSDQTYPEGTQAIYKCRPGYRSLGNVIMVCRKGEWVALNPLRKCQKRPCPNPGEIRNGQIDVPGGILFGATISFSCNTGYKLFGSTSSFCLISGSSVQWSDPLPECREIYCPAPPQIDNGIIQGERDHYGYRQSVTYACNKGFTMIGEHSIYCTVNNDEGEWSGPPPECRG

SEQ ID NO: 19 - protein, 189 aa, artificial sequence
EDCNELPPRRNTEILTGSWSDQTYPEGTQAIYKCRPGYRSLGNVIMVCRKGEWVALNPLRKCQKKSCPNPGEIRNGQIDVPGGILFGATISFSCNTGYKLFGSTSSFCLISGSSVQWSDPLPECREIYCPAPPQIDNGIIQGERDHYGYRQSVTYACNKGFTMIGEHSIYCTVNNDEGEWSGPPPECRG

SEQ ID NO: 20 - protein, 189 aa, artificial sequence
EDCNELPPRRNTEILTGSWSDQTYPEGTQAIYKCRPGYRSLGNIIMVCRKGEWVALNPLRKCQKKSCPNPGEIRNGQIDVPGGILFGATISFSCNTGYKLFGSTSSFCLISGSSVQWSDPLPECREIYCPAPPQIDNGIIQGERDHYGYRQSVTYACNKGFTMIGEHSIYCTVNNDEGEWSGPPPECRG

SEQ ID NO: 21 - protein, 189 aa, artificial sequence
EDCNELPPRRNTEILTGSWSDQTYPEGTQAIYKCRPGYRSLGNIIMVCRKGEWVALNPLRKCQKRPCPNPGEIRNGQIDVPGGILFGATISFSCNTGYKLFGSTSSFCLISGSSVQWSDPLPECREIYCPAPPQIDNGIIQGERDHYGYRQSVTYACNKGFTMIGEHSIYCTVNNDEGEWSGPPPECRG

SEQ ID NO: 22 - protein, 196 aa, artificial sequence
EDCNELPPRRNTEILTGSWSDQTYPEGTQAIYKCRPGYRSLGNVIMVCRKGEWVALNPLRKCQKRPCPNPGEIRNGQIDVPGGILFGATISFSCNTGYKLFGSTSSFCLISGSSVQWSDPLPECREIYCPAPPQIDNGIIQGERDHYGYRQSVTYACNKGFTMIGEHSIYCTVNNDEGEWSGPPPECRGGHHHHHH

SEQ ID NO: 23 - protein, 196 aa, artificial sequence
EDCNELPPRRNTEILTGSWSDQTYPEGTQAIYKCRPGYRSLGNVIMVCRKGEWVALNPLRKCQKKSCPNPGEIRNGQIDVPGGILFGATISFSCNTGYKLFGSTSSFCLISGSSVQWSDPLPECREIYCPAPPQIDNGIIQGERDHYGYRQSVTYACNKGFTMIGEHSIYCTVNNDEGEWSGPPPECRGGHHHHHH

SEQ ID NO: 24 - protein, 196 aa, artificial sequence
EDCNELPPRRNTEILTGSWSDQTYPEGTQAIYKCRPGYRSLGNIIMVCRKGEWVALNPLRKCQKKSCPNPGEIRNGQIDVPGGILFGATISFSCNTGYKLFGSTSSFCLISGSSVQWSDPLPECREIYCPAPPQIDNGIIQGERDHYGYRQSVTYACNKGFTMIGEHSIYCTVNNDEGEWSGPPPECRGGHHHHHH

SEQ ID NO: 25 - protein, 196 aa, artificial sequence
EDCNELPPRRNTEILTGSWSDQTYPEGTQAIYKCRPGYRSLGNIIMVCRKGEWVALNPLRKCQKRPCPNPGEIRNGQIDVPGGILFGATISFSCNTGYKLFGSTSSFCLISGSSVQWSDPLPECREIYCPAPPQIDNGIIQGERDHYGYRQSVTYACNKGFTMIGEHSIYCTVNNDEGEWSGPPPECRGGHHHHHH

SEQ ID NO: 26 - protein, 215 aa, artificial sequence
MGWSCIILFLVATATGVHSEDCNELPPRRNTEILTGSWSDQTYPEGTQAIYKCRPGYRSLGNVIMVCRKGEWVALNPLRKCQKRPCPNPGEIRNGQIDVPGGILFGATISFSCNTGYKLFGSTSSFCLISGSSVQWSDPLPECREIYCPAPPQIDNGIIQGERDHYGYRQSVTYACNKGFTMIGEHSIYCTVNNDEGEWSGPPPECRGGHHHHHH

SEQ ID NO: 27 - protein, 215 aa, artificial sequence
MGWSCIILFLVATATGVHSEDCNELPPRRNTEILTGSWSDQTYPEGTQAIYKCRPGYRSLGNVIMVCRKGEWVALNPLRKCQKKSCPNPGEIRNGQIDVPGGILFGATISFSCNTGYKLFGSTSSFCLISGSSVQWSDPLPECREIYCPAPPQIDNGIIQGERDHYGYRQSVTYACNKGFTMIGEHSIYCTVNNDEGEWSGPPPECRGGHHHHHH

SEQ ID NO: 28 - protein, 215 aa, artificial sequence
MGWSCIILFLVATATGVHSEDCNELPPRRNTEILTGSWSDQTYPEGTQAIYKCRPGYRSLGNIIMVCRKGEWVALNPLRKCQKKSCPNPGEIRNGQIDVPGGILFGATISFSCNTGYKLFGSTSSFCLISGSSVQWSDPLPECREIYCPAPPQIDNGIIQGERDHYGYRQSVTYACNKGFTMIGEHSIYCTVNNDEGEWSGPPPECRGGHHHHHH

SEQ ID NO: 29 - protein, 215 aa, artificial sequence
MGWSCIILFLVATATGVHSEDCNELPPRRNTEILTGSWSDQTYPEGTQAIYKCRPGYRSLGNIIMVCRKGEWVALNPLRKCQKRPCPNPGEIRNGQIDVPGGILFGATISFSCNTGYKLFGSTSSFCLISGSSVQWSDPLPECREIYCPAPPQIDNGIIQGERDHYGYRQSVTYACNKGFTMIGEHSIYCTVNNDEGEWSGPPPECRGGHHHHHH

SEQ ID NO: 30 - protein, 208 aa, artificial sequence
MGWSCIILFLVATATGVHSEDCNELPPRRNTEILTGSWSDQTYPEGTQAIYKCRPGYRSLGNVIMVCRKGEWVALNPLRKCQKRPCPNPGEIRNGQIDVPGGILFGATISFSCNTGYKLFGSTSSFCLISGSSVQWSDPLPECREIYCPAPPQIDNGIIQGERDHYGYRQSVTYACNKGFTMIGEHSIYCTVNNDEGEWSGPPPECRG

SEQ ID NO: 31 - protein, 208 aa, artificial sequence
MGWSCIILFLVATATGVHSEDCNELPPRRNTEILTGSWSDQTYPEGTQAIYKCRPGYRSLGNVIMVCRKGEWVALNPLRKCQKKSCPNPGEIRNGQIDVPGGILFGATISFSCNTGYKLFGSTSSFCLISGSSVQWSDPLPECREIYCPAPPQIDNGIIQGERDHYGYRQSVTYACNKGFTMIGEHSIYCTVNNDEGEWSGPPPECRG

SEQ ID NO: 32 - protein, 208 aa, artificial sequence
MGWSCIILFLVATATGVHSEDCNELPPRRNTEILTGSWSDQTYPEGTQAIYKCRPGYRSLGNIIMVCRKGEWVALNPLRKCQKKSCPNPGEIRNGQIDVPGGILFGATISFSCNTGYKLFGSTSSFCLISGSSVQWSDPLPECREIYCPAPPQIDNGIIQGERDHYGYRQSVTYACNKGFTMIGEHSIYCTVNNDEGEWSGPPPECRG

SEQ ID NO: 33 - protein, 208 aa, artificial sequence
MGWSCIILFLVATATGVHSEDCNELPPRRNTEILTGSWSDQTYPEGTQAIYKCRPGYRSLGNIIMVCRKGEWVALNPLRKCQKRPCPNPGEIRNGQIDVPGGILFGATISFSCNTGYKLFGSTSSFCLISGSSVQWSDPLPECREIYCPAPPQIDNGIIQGERDHYGYRQSVTYACNKGFTMIGEHSIYCTVNNDEGEWSGPPPECRG

SEQ ID NO: 34 - protein, 199 aa, artificial sequence
QCNAPEWLPFARPTNLTDEFEFPIGTYLKYECRPGYYGRPFSIICLKNSVWTGAKDRCRRKSCRNPPDPVNGMVHVIKDIQFGSQIKYSCTKGYRLIGSSSATCIISGNTVIWDNETPICDRIPCGLPPTITNGDFISTNRENFHYGSVVTYRCNPGSGGRKVFELVGEPSIYCTSNDDQVGIWSGPAPQCIGHHHHHH

SEQ ID NO: 35 - protein, 196 aa, artificial sequence
SCEVPTRLNSASLKQPYITQNYFPVGTVVEYECRPGYRREPSLSPKLTCLQNLKWSTAVEFCKKKSCPNPGEIRNGQIDVPGGILFGATISFSCNTGYKLFGSTSSFCLISGSSVQWSDPLPECREIYCPAPPQIDNGIIQGERDHYGYRQSVTYACNKGFTMIGEHSIYCTVNNDEGEWSGPPPECRGGHHHHHH

SEQ ID NO: 36 - protein, 313 aa, artificial sequence
EDCNELPPRRNTEILTGSWSDQTYPEGTQAIYKCRPGYRSLGNIIMVCRKGEWVALNPLRKCQKRPCGHPGDTPFGTFTLTGGNVFEYGVKAVYTCNEGYQLLGEINYRECDTDGWTNDIPICEVVKCLPVTAPENGKIVSSAMEPDREYHFGQAVRFVCNSGYKIEGDEEMHCSDDGFWSKEKPKCVEISCKSPDVINGSPISQKIIYKENERFQYKCNMGYEYSERGDAVCTESGWRPLPSCEEKSCDNPYIPNGDYSPLRIKHRTGDEITYQCRNGFYPATRGNTAKCTSTGWIPAPRCTLKPGHHHHHH

SEQ ID NO: 37 - protein, 193 aa, artificial sequence
GHCQAPDHFLFAKLKTQTNASDFPIGTSLKYECRPEYYGRPFSITCLDNLVWSSPKDVCKRKSCPNPGEIRNGQIDVPGGILFGATISFSCNTGYKLFGSTSSFCLISGSSVQWSDPLPECREIYCPAPPQIDNGIIQGERDHYGYRQSVTYACNKGFTMIGEHSIYCTVNNDEGEWSGPPPECRGGHHHHHH

SEQ ID NO: 38 - protein, 1658 aa, artificial sequence
QEQTYVISAPKIFRVGASENIVIQVYGYTEAFDATISIKSYPDKKFSYSSGHVHLSSENKFQNSAILTIQPKQLPGGQNPVSYVYLEVVSKHFSKSKRMPITYDNGFLFIHTDKPVYTPDQSVKVRVYSLNDDLKPAKRETVLTFIDPEGSEVDMVEEIDHIGIISFPDFKIPSNPRYGMWTIKAKYKEDFSTTGTAYFEVKEYVLPHFSVSIEPEYNFIGYKNFKNFEITIKARYFYNKVVTEADVYITFGIREDLKDDQKEMMQTAMQNTMLINGIAQVTFDSETAVKELSYYSLEDLNNKYLYIAVTVIESTGGFSEEAEIPGIKYVLSPYKLNLVATPLFLKPGIPYPIKVQVKDSLDQLVGGVPVTLNAQTIDVNQETSDLDPSKSVTRVDDGVASFVLNLPSGVTVLEFNVKTDAPDLPEENQAREGYRAIAYSSLSQSYLYIDWTDNHKALLVGEHLNIIVTPKSPYIDKITHYNYLILSKGKIIHFGTREKFSDASYQSINIPVTQNMVPSSRLLVYYIVTGEQTAELVSDSVWLNIEEKCGNQLQVHLSPDADAYSPGQTVSLNMATGMDSWVALAAVDSAVYGVQRGAKKPLERVFQFLEKSDLGCGAGGGLNNANVFHLAGLTFLTNANADDSQENDEPCKEILRPRRTLQKKIEEIAAKYKHSVVKKCCYDGACVNNDETCEQRAARISLGPRCIKAFTECCVVASQLRANISHKDMQLGRLHMKTLLPVSKPEIRSYFPESWLWEVHLVPRRKQLQFALPDSLTTWEIQGVGISNTGICVADTVKAKVFKDVFLEMNIPYSVVRGEQIQLKGTVYNYRTSGMQFCVKMSAVEGICTSESPVIDHQGTKSSKCVRQKVEGSSSHLVTFTVLPLEIGLHNINFSLETWFGKEILVKTLRVVPEGVKRESYSGVTLDPRGIYGTISRRKEFPYRIPLDLVPKTEIKRILSVKGLLVGEILSAVLSQEGINILTHLPKGSAEAELMSVVPVFYVFHYLETGNHWNIFHSDPLIEKQKLKKKLKEGMLSIMSYRNADYSYSVWKGGSASTWLTAFALRVLGQVNKYVEQNQNSICNSLLWLVENYQLDNGSFKENSQYQPIKLQGTLPVEARENSLYLTAFTVIGIRKAFDICPLVKIDTALIKADNFLLENTLPAQSTFTLAISAYALSLGDKTHPQFRSIVSALKREALVKGNPPIYRFWKDNLQHKDSSVPNTGTARMVETTAYALLTSLNLKDINYVNPVIKWLSEEQRYGGGFYSTQDTINAIEGLTEYSLLVKQLRLSMDIDVSYKHKGALHNYKMTDKNFLGRPVEVLLNDDLIVSTGFGSGLATVHVTTVVHKTSTSEEVCSFYLKIDTQDIEASHYRGYGNSDYKRIVACASYKPSREESSSGSSHAVMDISLPTGISANEEDLKALVEGVDQLFTDYQIKDGHVILQLNSIPSSDFLCVRFRIFELFEVGFLSPATFTVYEYHRPDKQCTMFYSTSNIKIQKVCEGAACKCVEADCGQMQEELDLTISAETRKQTACKPEIAYAYKVSITSITVENVFVKYKATLLDIYKTGEAVAEKDSEITFIKKVTCTNAELVKGRQYLIMGKEALQIKYNFSFRYIYPLDSLTWIEYWPRDTTCSSCQAFLANLDEFAEDIFLNGC

SEQ ID NO: 39 - protein, 122 aa, artificial sequence
QVQLVQSGAEVKKPGASVKVSCKASGYTFTNYGMNWVRQAPGQGLEWMGWINTYTGEPTYADDFKGRFTFTLDTSTSTAYLELSSLRSEDTAVYYCARTKVPHYFAYAMDYWGQGTLVTVSS

SEQ ID NO: 40 - protein, 5 aa, artificial sequence
NYGMN

SEQ ID NO: 41 - protein, 17 aa, artificial sequence
WINTYTGEPTYADDFKG

SEQ ID NO: 42 - protein, 13 aa, artificial sequence
TKVPHYFAYAMDY

SEQ ID NO: 43 - protein, 327 aa, artificial sequence
ASTKGPSVFPLAPCSRSTSESTAALGCLVKDYFPEPVTVSWNSGALTSGVHTFPAVLQSSGLYSLSSVVTVPSSSLGTKTYTCNVDHKPSNTKVDKRVESKYGPPCPPCPAPEFLGGPSVFLFPPKPKDTLMISRTPEVTCVVVDVSQEDPEVQFNWYVDGVEVHNAKTKPREEQFNSTYRVVSVLTVLHQDWLNGKEYKCKVSNKGLPSSIEKTISKAKGQPREPQVYTLPPSQEEMTKNQVSLTCLVKGFYPSDIAVEWESNGQPENNYKTTPPVLDSDGSFFLYSRLTVDKSRWQEGNVFSCSVLHEALHAHYTQKSLSLSLGK

SEQ ID NO: 44 - protein, 449 aa, artificial sequence
QVQLVQSGAEVKKPGASVKVSCKASGYTFTNYGMNWVRQAPGQGLEWMGWINTYTGEPTYADDFKGRFTFTLDTSTSTAYLELSSLRSEDTAVYYCARTKVPHYFAYAMDYWGQGTLVTVSSASTKGPSVFPLAPCSRSTSESTAALGCLVKDYFPEPVTVSWNSGALTSGVHTFPAVLQSSGLYSLSSVVTVPSSSLGTKTYTCNVDHKPSNTKVDKRVESKYGPPCPPCPAPEFLGGPSVFLFPPKPKDTLMISRTPEVTCVVVDVSQEDPEVQFNWYVDGVEVHNAKTKPREEQFNSTYRVVSVLTVLHQDWLNGKEYKCKVSNKGLPSSIEKTISKAKGQPREPQVYTLPPSQEEMTKNQVSLTCLVKGFYPSDIAVEWESNGQPENNYKTTPPVLDSDGSFFLYSRLTVDKSRWQEGNVFSCSVLHEALHAHYTQKSLSLSLGK

SEQ ID NO: 45 - protein, 111 aa, artificial sequence
DIVLTQSPSSLSASVGDRVTITCKASQSVDYHGDSYLNWYQQKPGKPPKLLIYAASNLESGIPSRFSGSGSGTDFTLTISSLQPEDFATYYCQQSNEDPSTFGGGTKLEIK

SEQ ID NO: 46 - protein, 15 aa, artificial sequence
KASQSVDYHGDSYLN

SEQ ID NO: 47 - protein, 7 aa, artificial sequence
AASNLES

SEQ ID NO: 48 - protein, 9 aa, artificial sequence
QQSNEDPST

SEQ ID NO: 49 - protein, 107 aa, artificial sequence [sequence omitted]

SEQ ID NO: 50 - protein, 218 aa, artificial sequence
DIVLTQSPSSLSASVGDRVTITCKASQSVDYHGDSYLNWYQQKPGKPPKLLIYAASNLESGIPSRFSGSGSGTDFTLTISSLQPEDFATYYCQQSNEDPSTFGGGTKLEIKRTVAAPSVFIFPPSDEQLKSGTASVVCLLNNFYPREAKVQWKVDNALQSGNSQESVTEQDSKDSTYSLSSTLTLSKADYEKHKVYACEVTHQGLSSPVTKSFNRGEC

SEQ ID NO: 51 - protein, 758 aa, artificial sequence
QVQLVQSGAEVKKPGASVKVSCKASGYTFTNYGMNWVRQAPGQGLEWMGWINTYTGEPTYADDFKGRFTFTLDTSTSTAYLELSSLRSEDTAVYYCARTKVPHYFAYAMDYWGQGTLVTVSSASTKGPSVFPLAPCSRSTSESTAALGCLVKDYFPEPVTVSWNSGALTSGVHTFPAVLQSSGLYSLSSVVTVPSSSLGTKTYTCNVDHKPSNTKVDKRVESKYGPPCPPCPAPEFLGGPSVFLFPPKPKDTLMISRTPEVTCVVVDVSQEDPEVQFNWYVDGVEVHNAKTKPREEQFNSTYRVVSVLTVLHQDWLNGKEYKCKVSNKGLPSSIEKTISKAKGQPREPQVYTLPPSQEEMTKNQVSLTCLVKGFYPSDIAVEWESNGQPENNYKTTPPVLDSDGSFFLYSRLTVDKSRWQEGNVFSCSVLHEALHAHYTQKSLSLSLGKGSGEDCNELPPRRNTEILTGSWSDQTYPEGTQAIYKCRPGYRSLGNVIMVCRKGEWVALNPLRKCQKRPCGHPGDTPFGTFTLTGGNVFEYGVKAVYTCNEGYQLLGEINYRECDTDGWTNDIPICEVVKCLPVTAPENGKIVSSAMEPDREYHFGQAVRFVCNSGYKIEGDEEMHCSDDGFWSKEKPKCVEISCKSPDVINGSPISQKIIYKENERFQYKCNMGYEYSERGDAVCTESGWRPLPSCEEKSCDNPYIPNGDYSPLRIKHRTGDEITYQCRNGFYPATRGNTAKCTSTGWIPAPRCTLKP

SEQ ID NO: 52 - protein, 638 aa, artificial sequence
QVQLVQSGAEVKKPGASVKVSCKASGYTFTNYGMNWVRQAPGQGLEWMGWINTYTGEPTYADDFKGRFTFTLDTSTSTAYLELSSLRSEDTAVYYCARTKVPHYFAYAMDYWGQGTLVTVSSASTKGPSVFPLAPCSRSTSESTAALGCLVKDYFPEPVTVSWNSGALTSGVHTFPAVLQSSGLYSLSSVVTVPSSSLGTKTYTCNVDHKPSNTKVDKRVESKYGPPCPPCPAPEFLGGPSVFLFPPKPKDTLMISRTPEVTCVVVDVSQEDPEVQFNWYVDGVEVHNAKTKPREEQFNSTYRVVSVLTVLHQDWLNGKEYKCKVSNKGLPSSIEKTISKAKGQPREPQVYTLPPSQEEMTKNQVSLTCLVKGFYPSDIAVEWESNGQPENNYKTTPPVLDSDGSFFLYSRLTVDKSRWQEGNVFSCSVLHEALHAHYTQKSLSLSLGKGSGGHCQAPDHFLFAKLKTQTNASDFPIGTSLKYECRPEYYGRPFSITCLDNLVWSSPKDVCKRKSCPNPGEIRNGQIDVPGGILFGATISFSCNTGYKLFGSTSSFCLISGSSVQWSDPLPECREIYCPAPPQIDNGIIQGERDHYGYRQSVTYACNKGFTMIGEHSIYCTVNNDEGEWSGPPPECRG

SEQ ID NO: 53 - protein, 643 aa, artificial sequence
QVQLVQSGAEVKKPGASVKVSCKASGYTFTNYGMNWVRQAPGQGLEWMGWINTYTGEPTYADDFKGRFTFTLDTSTSTAYLELSSLRSEDTAVYYCARTKVPHYFAYAMDYWGQGTLVTVSSASTKGPSVFPLAPCSRSTSESTAALGCLVKDYFPEPVTVSWNSGALTSGVHTFPAVLQSSGLYSLSSVVTVPSSSLGTKTYTCNVDHKPSNTKVDKRVESKYGPPCPPCPAPEFLGGPSVFLFPPKPKDTLMISRTPEVTCVVVDVSQEDPEVQFNWYVDGVEVHNAKTKPREEQFNSTYRVVSVLTVLHQDWLNGKEYKCKVSNKGLPSSIEKTISKAKGQPREPQVYTLPPSQEEMTKNQVSLTCLVKGFYPSDIAVEWESNGQPENNYKTTPPVLDSDGSFFLYSRLTVDKSRWQEGNVFSCSVLHEALHAHYTQKSLSLSLGKGGGGSSCEVPTRLNSASLKQPYITQNYFPVGTVVEYECRPGYRREPSLSPKLTCLQNLKWSTAVEFCKKKSCPNPGEIRNGQIDVPGGILFGATISFSCNTGYKLFGSTSSFCLISGSSVQWSDPLPECREIYCPAPPQIDNGIIQGERDHYGYRQSVTYACNKGFTMIGEHSIYCTVNNDEGEWSGPPPECRG

SEQ ID NO: 54 - protein, 641 aa, artificial sequence
QVQLVQSGAEVKKPGASVKVSCKASGYTFTNYGMNWVRQAPGQGLEWMGWINTYTGEPTYADDFKGRFTFTLDTSTSTAYLELSSLRSEDTAVYYCARTKVPHYFAYAMDYWGQGTLVTVSSASTKGPSVFPLAPCSRSTSESTAALGCLVKDYFPEPVTVSWNSGALTSGVHTFPAVLQSSGLYSLSSVVTVPSSSLGTKTYTCNVDHKPSNTKVDKRVESKYGPPCPPCPAPEFLGGPSVFLFPPKPKDTLMISRTPEVTCVVVDVSQEDPEVQFNWYVDGVEVHNAKTKPREEQFNSTYRVVSVLTVLHQDWLNGKEYKCKVSNKGLPSSIEKTISKAKGQPREPQVYTLPPSQEEMTKNQVSLTCLVKGFYPSDIAVEWESNGQPENNYKTTPPVLDSDGSFFLYSRLTVDKSRWQEGNVFSCSVLHEALHAHYTQKSLSLSLGKGSGEDCNELPPRRNTEILTGSWSDQTYPEGTQAIYKCRPGYRSLGNVIMVCRKGEWVALNPLRKCQKKSCPNPGEIRNGQIDVPGGILFGATISFSCNTGYKLFGSTSSFCLISGSSVQWSDPLPECREIYCPAPPQIDNGIIQGERDHYGYRQSVTYACNKGFTMIGEHSIYCTVNNDEGEWSGPPPECRG

SEQ ID NO: 55 - protein, 641 aa, artificial sequence
QVQLVQSGAEVKKPGASVKVSCKASGYTFTNYGMNWVRQAPGQGLEWMGWINTYTGEPTYADDFKGRFTFTLDTSTSTAYLELSSLRSEDTAVYYCARTKVPHYFAYAMDYWGQGTLVTVSSASTKGPSVFPLAPCSRSTSESTAALGCLVKDYFPEPVTVSWNSGALTSGVHTFPAVLQSSGLYSLSSVVTVPSSSLGTKTYTCNVDHKPSNTKVDKRVESKYGPPCPPCPAPEFLGGPSVFLFPPKPKDTLMISRTPEVTCVVVDVSQEDPEVQFNWYVDGVEVHNAKTKPREEQFNSTYRVVSVLTVLHQDWLNGKEYKCKVSNKGLPSSIEKTISKAKGQPREPQVYTLPPSQEEMTKNQVSLTCLVKGFYPSDIAVEWESNGQPENNYKTTPPVLDSDGSFFLYSRLTVDKSRWQEGNVFSCSVLHEALHAHYTQKSLSLSLGKGSGEDCNELPPRRNTEILTGSWSDQTYPEGTQAIYKCRPGYRSLGNIIMVCRKGEWVALNPLRKCQKKSCPNPGEIRNGQIDVPGGILFGATISFSCNTGYKLFGSTSSFCLISGSSVQWSDPLPECREIYCPAPPQIDNGIIQGERDHYGYRQSVTYACNKGFTMIGEHSIYCTVNNDEGEWSGPPPECRG

SEQ ID NO: 56 - protein, 641 aa, artificial sequence
QVQLVQSGAEVKKPGASVKVSCKASGYTFTNYGMNWVRQAPGQGLEWMGWINTYTGEPTYADDFKGRFTFTLDTSTSTAYLELSSLRSEDTAVYYCARTKVPHYFAYAMDYWGQGTLVTVSSASTKGPSVFPLAPCSRSTSESTAALGCLVKDYFPEPVTVSWNSGALTSGVHTFPAVLQSSGLYSLSSVVTVPSSSLGTKTYTCNVDHKPSNTKVDKRVESKYGPPCPPCPAPEFLGGPSVFLFPPKPKDTLMISRTPEVTCVVVDVSQEDPEVQFNWYVDGVEVHNAKTKPREEQFNSTYRVVSVLTVLHQDWLNGKEYKCKVSNKGLPSSIEKTISKAKGQPREPQVYTLPPSQEEMTKNQVSLTCLVKGFYPSDIAVEWESNGQPENNYKTTPPVLDSDGSFFLYSRLTVDKSRWQEGNVFSCSVLHEALHAHYTQKSLSLSLGKGSGEDCNELPPRRNTEILTGSWSDQTYPEGTQAIYKCRPGYRSLGNVIMVCRKGEWVALNPLRKCQKRPCPNPGEIRNGQIDVPGGILFGATISFSCNTGYKLFGSTSSFCLISGSSVQWSDPLPECREIYCPAPPQIDNGIIQGERDHYGYRQSVTYACNKGFTMIGEHSIYCTVNNDEGEWSGPPPECRG

SEQ ID NO: 57 - protein, 639 aa, artificial sequence
QVQLVQSGAEVKKPGASVKVSCKASGYTFTNYGMNWVRQAPGQGLEWMGWINTYTGEPTYADDFKGRFTFTLDTSTSTAYLELSSLRSEDTAVYYCARTKVPHYFAYAMDYWGQGTLVTVSSASTKGPSVFPLAPCSRSTSESTAALGCLVKDYFPEPVTVSWNSGALTSGVHTFPAVLQSSGLYSLSSVVTVPSSSLGTKTYTCNVDHKPSNTKVDKRVESKYGPPCPPCPAPEFLGGPSVFLFPPKPKDTLMISRTPEVTCVVVDVSQEDPEVQFNWYVDGVEVHNAKTKPREEQFNSTYRVVSVLTVLHQDWLNGKEYKCKVSNKGLPSSIEKTISKAKGQPREPQVYTLPPSQEEMTKNQVSLTCLVKGFYPSDIAVEWESNGQPENNYKTTPPVLDSDGSFFLYSRLTVDKSRWQEGNVFSCSVLHEALHAHYTQKSLSLSLGKGEDCNELPPRRNTEILTGSWSDQTYPEGTQAIYKCRPGYRSLGNIIMVCRKGEWVALNPLRKCQKKSCPNPGEIRNGQIDVPGGILFGATISFSCNTGYKLFGSTSSFCLISGSSVQWSDPLPECREIYCPAPPQIDNGIIQGERDHYGYRQSVTYACNKGFTMIGEHSIYCTVNNDEGEWSGPPPECRG

SEQ ID NO: 58 - protein, 638 aa, artificial sequence
QVQLVQSGAEVKKPGASVKVSCKASGYTFTNYGMNWVRQAPGQGLEWMGWINTYTGEPTYADDFKGRFTFTLDTSTSTAYLELSSLRSEDTAVYYCARTKVPHYFAYAMDYWGQGTLVTVSSASTKGPSVFPLAPCSRSTSESTAALGCLVKDYFPEPVTVSWNSGALTSGVHTFPAVLQSSGLYSLSSVVTVPSSSLGTKTYTCNVDHKPSNTKVDKRVESKYGPPCPPCPAPEFLGGPSVFLFPPKPKDTLMISRTPEVTCVVVDVSQEDPEVQFNWYVDGVEVHNAKTKPREEQFNSTYRVVSVLTVLHQDWLNGKEYKCKVSNKGLPSSIEKTISKAKGQPREPQVYTLPPSQEEMTKNQVSLTCLVKGFYPSDIAVEWESNGQPENNYKTTPPVLDSDGSFFLYSRLTVDKSRWQEGNVFSCSVLHEALHAHYTQKSLSLSLGKEDCNELPPRRNTEILTGSWSDQTYPEGTQAIYKCRPGYRSLGNIIMVCRKGEWVALNPLRKCQKKSCPNPGEIRNGQIDVPGGILFGATISFSCNTGYKLFGSTSSFCLISGSSVQWSDPLPECREIYCPAPPQIDNGIIQGERDHYGYRQSVTYACNKGFTMIGEHSIYCTVNNDEGEWSGPPPECRG

SEQ ID NO: 59 - protein, 217 aa, artificial sequence
APEFLGGPSVFLFPPKPKDTLMISRTPEVTCVVVDVSQEDPEVQFNWYVDGVEVHNAKTKPREEQFNSTYRVVSVLTVLHQDWLNGKEYKCKVSNKGLPSSIEKTISKAKGQPREPQVYTLPPSQEEMTKNQVSLTCLVKGFYPSDIAVEWESNGQPENNYKTTPPVLDSDGSFFLYSRLTVDKSRWQEGNVFSCSVLHEALHAHYTQKSLSLSLGK

SEQ ID NO: 60 - protein, 198 aa, artificial sequence
EDCNELPPRRNTEILTGSWSDQTYPEGTQAIYKCRPGYRSLGNIIMVCRKGEWVALNPLRKCQKRPCGHPGDTPFGTFTLTGGNVFEYGVKAVYTCNEGYQLLGEINYRECDTDGWTNDIPICEVVKCLPVTAPENGKIVSSAMEPDREYHFGQAVRFVCNSGYKIEGDEEMHCSDDGFWSKEKPKCVEISGHHHHHH

SEQ ID NO: 61 - protein, 260 aa, artificial sequence
DCGLPPDVPNAQPALEGRTSFPEDTVITYKCEESFVKIPGEKDSVICLKGSQWSDIEEFCNRSCEVPTRLNSASLKQPYITQNYFPVGTVVEYECRPGYRREPSLSPKLTCLQNLKWSTAVEFCKKKSCPNPGEIRNGQIDVPGGILFGATISFSCNTGYKLFGSTSSFCLISGSSVQWSDPLPECREIYCPAPPQIDNGIIQGERDHYGYRQSVTYACNKGFTMIGEHSIYCTVNNDEGEWSGPPPECRGKSGHHHHHH

SEQ ID NO: 62-67 - skipped (6 entries)

SEQ ID NO: 68 - protein, 5 aa, artificial sequence
  REPEAT 1..5: note = REPEAT=1-10, e.g., 1, 2, 3, 4, 5 or 6
GGGGS

SEQ ID NO: 69 - skipped

SEQ ID NO: 70 - protein, 5 aa, artificial sequence
GGGGS